European Patent Application EP 4 272 757 A2, published November 8, 2023. Title: MODIFIED NK-92 CELLS FOR TREATING CANCER. Applicant: NANTKWEST, INC. The sequence listing filed with the application follows.

SEQUENCE LISTING (13 sequences)

SEQ ID NO: 1 - protein, 236 aa, synthetic construct
  REGION 1..236: note = synthetic Low Affinity Immunoglobulin Gamma Fc Region Receptor III-A amino acid sequence (mature form)
RTEDLPKAVVFLEPQWYRVLEKDSVTLKCQGAYSPEDNSTQWFHNESLISSQASSYFIDAATVDDSGEYRCQTNLSTLSDPVQLEVHIGWLLLQAPRWVFKEEDPIHLRCHSWKNTALHKVTYLQNGKGRKYFHHNSDFYIPKATLKDSGSYFCRGLFGSKNVSSETVNITITQGLAVSTISSFFPPGYQVSFCLVMVLLFAVDTGLYFSVKTNIRSSTRDWKDHKFKWRKDPQDK

SEQ ID NO: 2 - protein, 236 aa, synthetic construct
  REGION 1..236: note = synthetic High Affinity Variant F158V Immunoglobulin Gamma Fc Region Receptor III-A amino acid sequence (mature form)
RTEDLPKAVVFLEPQWYRVLEKDSVTLKCQGAYSPEDNSTQWFHNESLISSQASSYFIDAATVDDSGEYRCQTNLSTLSDPVQLEVHIGWLLLQAPRWVFKEEDPIHLRCHSWKNTALHKVTYLQNGKGRKYFHHNSDFYIPKATLKDSGSYFCRGLVGSKNVSSETVNITITQGLAVSTISSFFPPGYQVSFCLVMVLLFAVDTGLYFSVKTNIRSSTRDWKDHKFKWRKDPQDK

SEQ ID NO: 3 - protein, 254 aa, synthetic construct
  REGION 1..254: note = synthetic Low Affinity Immunoglobulin Gamma Fc Region Receptor III-A amino acid sequence (precursor form)
MWQLLLPTALLLLVSAGMRTEDLPKAVVFLEPQWYRVLEKDSVTLKCQGAYSPEDNSTQWFHNESLISSQASSYFIDAATVDDSGEYRCQTNLSTLSDPVQLEVHIGWLLLQAPRWVFKEEDPIHLRCHSWKNTALHKVTYLQNGKGRKYFHHNSDFYIPKATLKDSGSYFCRGLFGSKNVSSETVNITITQGLAVSTISSFFPPGYQVSFCLVMVLLFAVDTGLYFSVKTNIRSSTRDWKDHKFKWRKDPQDK

SEQ ID NO: 4 - protein, 254 aa, synthetic construct
  REGION 1..254: note = synthetic High Affinity Variant Immunoglobulin Gamma Fc Region Receptor III-A amino acid sequence (precursor form)
MWQLLLPTALLLLVSAGMRTEDLPKAVVFLEPQWYRVLEKDSVTLKCQGAYSPEDNSTQWFHNESLISSQASSYFIDAATVDDSGEYRCQTNLSTLSDPVQLEVHIGWLLLQAPRWVFKEEDPIHLRCHSWKNTALHKVTYLQNGKGRKYFHHNSDFYIPKATLKDSGSYFCRGLVGSKNVSSETVNITITQGLAVSTISSFFPPGYQVSFCLVMVLLFAVDTGLYFSVKTNIRSSTRDWKDHKFKWRKDPQDK

SEQ ID NO: 5 - DNA, 765 bp, synthetic construct
  misc_feature 1..765: note = synthetic Polynucleotide Encoding the Low Affinity Immunoglobulin Gamma Fc Region Receptor III-A (Precursor)
  source 1..765: mol_type = other DNA
atgtggcagctgctcctcccaactgctctgctacttctagtttcagctggcatgcggactgaagatctcccaaaggctgtggtgttcctggagcctcaatggtacagggtgctcgagaaggacagtgtgactctgaagtgccagggagcctactcccctgaggacaattccacacagtggtttcacaatgagagcctcatctcaagccaggcctcgagctacttcattgacgctgccacagtcgacgacagtggagagtacaggtgccagacaaacctctccaccctcagtgacccggtgcagctagaagtccatatcggctggctgttgctccaggcccctcggtgggtgttcaaggaggaagaccctattcacctgaggtgtcacagctggaagaacactgctctgcataaggtcacatatttacagaatggcaaaggcaggaagtattttcatcataattctgacttctacattccaaaagccacactcaaagacagcggctcctacttctgcagggggctttttgggagtaaaaatgtgtcttcagagactgtgaacatcaccatcactcaaggtttggcagtgtcaaccatctcatcattctttccacctgggtaccaagtctctttctgcttggtgatggtactcctttttgcagtggacacaggactatatttctctgtgaagacaaacattcgaagctcaacaagagactggaaggaccataaatttaaatggagaaaggaccctcaagacaaatga

SEQ ID NO: 6 - protein, 153 aa, synthetic construct
  REGION 1..153: note = synthetic polypeptide - Wild-Type IL-2
MYRMQLLSCIALSLALVTNSAPTSSSTKKTQLQLEHLLLDLQMILNGINNYKNPKLTRMLTFKFYMPKKATELKHLQCLEEELKPLEEVLNLAQSKNFHLRPRDLISNINVIVLELKGSETTFMCEYADETATIVEFLNRWITFCQSIISTLT

SEQ ID NO: 7 - protein, 160 aa, synthetic construct
  REGION 1..160: note = synthetic polypeptide IL-2-ER
MYRMQLLSCIALSLALVTNSAPTSSSTKKTQLQLEHLLLDLQMILNGINNYKNPKLTRMLTFKFYMPKKATELKHLQCLEEELKPLEEVLNLAQSKNFHLRPRDLISNINVIVLELKGSETTFMCEYADETATIVEFLNRWITFCQSIISTLTGSEKDEL

SEQ ID NO: 8 - DNA, 1455 bp, synthetic construct
  misc_feature 1..1455: note = synthetic CD19-CAR DNA sequence
  source 1..1455: mol_type = other DNA
cccgggaattcgccaccatggactggatctggcggatcctgttcctcgtgggagccgccacaggcgcccattctgcccagcccgccgacatccagatgacccagaccaccagcagcctgagcgccagcctgggcgacagagtgaccatcagctgccgggccagccaggacatcagcaagtacctgaactggtatcagcagaaacccgacggcaccgtgaagctgctgatctaccacaccagccggctgcacagcggcgtgcccagcagattttctggcagcggcagcggcaccgactacagcctgaccatctccaacctggaacaggaagatatcgctacctacttctgtcagcaaggcaacaccctgccctacaccttcggcggaggcaccaagctggaactgaagagaggcggcggaggctctggtggaggcggatctgggggcggaggaagtggcgggggaggatctgaagtgcagctgcagcagagcggccctggcctggtggcccctagccagagcctgtccgtgacctgtaccgtgtccggcgtgtccctgcccgactacggcgtgtcctggatccggcagccccccagaaagggcctggaatggctgggcgtgatctggggcagcgagacaacctactacaacagcgccctgaagtcccggctgaccatcatcaaggacaacagcaagagccaggtgttcctgaagatgaacagcctgcagaccgacgacaccgccatctactactgcgccaagcactactactacggcggcagctacgccatggactactggggccagggcaccaccgtgaccgtgtccagcgccctgtccaacagcatcatgtacttcagccacttcgtgcccgtgtttctgcccgccaagcccaccaccacccctgcccctagacctcccaccccagccccaacaatcgccagccagcctctgtccctgcggcccgaagctagcagacctgctgccggcggagccgtgcacaccagaggcctggaccccaagctgtgctacctgctggacggcatcctgttcatctatggcgtgatcctgaccgccctgttcctgagagtgaagttcagcagaagcgccgacgcccctgcctaccagcagggccagaaccagctgtacaacgagctgaacctgggcagacgggaagagtacgacgtgctggacaagcggagaggcagggaccccgagatgggcggcaagcccagacggaagaacccccaggaaggcctgtataacgaactgcagaaagacaagatggccgaggcctacagcgagatcggcatgaagggcgagcggcggaggggcaagggccacgatggactgtaccagggcctgagcaccgccaccaaggacacctacgacgccctgcacatgcaggccctgccccccagatgacagccagggcatttctccctcgagcggccgc

SEQ ID NO: 9 - protein, 468 aa, synthetic construct
  REGION 1..468: note = synthetic CD19-CAR amino acids sequence
MDWIWRILFLVGAATGAHSAQPADIQMTQTTSSLSASLGDRVTISCRASQDISKYLNWYQQKPDGTVKLLIYHTSRLHSGVPSRFSGSGSGTDYSLTISNLEQEDIATYFCQQGNTLPYTFGGGTKLELKRGGGGSGGGGSGGGGSGGGGSEVQLQQSGPGLVAPSQSLSVTCTVSGVSLPDYGVSWIRQPPRKGLEWLGVIWGSETTYYNSALKSRLTIIKDNSKSQVFLKMNSLQTDDTAIYYCAKHYYYGGSYAMDYWGQGTTVTVSSALSNSIMYFSHFVPVFLPAKPTTTPAPRPPTPAPTIASQPLSLRPEASRPAAGGAVHTRGLDPKLCYLLDGILFIYGVILTALFLRVKFSRSADAPAYQQGQNQLYNELNLGRREEYDVLDKRRGRDPEMGGKPRRKNPQEGLYNELQKDKMAEAYSEIGMKGERRRGKGHDGLYQGLSTATKDTYDALHMQALPPR

SEQ ID NO: 10 - DNA, 1437 bp, synthetic construct
  misc_feature 1..1437: note = synthetic CD33-CAR DNA sequence
  source 1..1437: mol_type = other DNA
cccgggaattcgccaccatggactggatctggcggatcctgttcctcgtgggagccgccacaggcgcccattctgcccagcccgccgacatccagatgacccagagccctagcagcctgagcgccagcgtgggcgacagagtgaccatcacctgtcgggccagcgagagcgtggacaactacggcatcagcttcatgaactggttccagcagaagcccggcaaggcccccaagctgctgatctacgccgccagcaatcagggcagcggcgtgcccagcagattcagcggctctggcagcggcaccgacttcaccctgaccatcagcagcctgcagcccgacgacttcgccacctactactgccagcagagcaaagaggtgccctggaccttcggccagggcaccaaggtggaaatcaagggcggaggcggcagcggaggtggaggaagtggcggcggaggatctcaggtgcagctggtgcagtctggcgccgaagtgaagaaacccggcagcagcgtgaaggtgtcctgcaaggccagcggctacaccttcaccgactacaacatgcactgggtccgccaggccccaggccagggactggaatggatcggctacatctacccctacaacggcggcaccggctacaaccagaagttcaagagcaaggccaccatcaccgccgacgagagcaccaacaccgcctacatggaactgagcagcctgcggagcgaggacaccgccgtgtactactgcgccagaggcagacccgccatggactactggggccagggaaccctggtgacagtgtccagcgccctgagcaacagcatcatgtacttcagccacttcgtgcccgtgtttctgcccgccaagcccaccaccacccctgcccctagacctcccaccccagccccaacaatcgccagccagcctctgtccctgcggcccgaagctagcagacctgctgccggcggagccgtgcacaccagaggcctggaccccaagctgtgctacctgctggacggcatcctgttcatctacggcgtgatcctgaccgccctgttcctgagagtgaagttcagcagaagcgccgacgcccctgcctaccagcagggccagaaccagctgtacaacgagctgaacctgggcagacgggaagagtacgacgtgctggacaagcggagaggcagggaccccgagatgggcggcaagcccagacggaagaacccccaggaaggcctgtataacgaactgcagaaagacaagatggccgaggcctacagcgagatcggcatgaagggcgagcggcggaggggcaagggccacgatggactgtaccagggcctgagcaccgccaccaaggacacctacgacgccctgcacatgcaggccctgccccccagatgacagccagggcatttctccctcgagcggccgc

SEQ ID NO: 11 - protein, 462 aa, synthetic construct
  REGION 1..462: note = synthetic CD33-CAR amino acid sequence
MDWIWRILFLVGAATGAHSAQPADIQMTQSPSSLSASVGDRVTITCRASESVDNYGISFMNWFQQKPGKAPKLLIYAASNQGSGVPSRFSGSGSGTDFTLTISSLQPDDFATYYCQQSKEVPWTFGQGTKVEIKGGGGSGGGGSGGGGSQVQLVQSGAEVKKPGSSVKVSCKASGYTFTDYNMHWVRQAPGQGLEWIGYIYPYNGGTGYNQKFKSKATITADESTNTAYMELSSLRSEDTAVYYCARGRPAMDYWGQGTLVTVSSALSNSIMYFSHFVPVFLPAKPTTTPAPRPPTPAPTIASQPLSLRPEASRPAAGGAVHTRGLDPKLCYLLDGILFIYGVILTALFLRVKFSRSADAPAYQQGQNQLYNELNLGRREEYDVLDKRRGRDPEMGGKPRRKNPQEGLYNELQKDKMAEAYSEIGMKGERRRGKGHDGLYQGLSTATKDTYDALHMQALPPR

SEQ ID NO: 12 - DNA, 1509 bp, synthetic construct
  misc_feature 1..1509: note = synthetic CSPG4-CAR DNA sequence
  source 1..1509: mol_type = other DNA
cccgggaattcgccaccatggactggatctggcgcatcctcttcctcgtcggcgctgctaccggcgctcattcggcccagccggccgatatcgagctcacccaatctccaaaattcatgtccacatcagtaggagacagggtcagcgtcacctgcaaggccagtcagaatgtggatactaatgtagcgtggtatcaacaaaaaccagggcaatctcctgaaccactgcttttctcggcatcctaccgttacactggagtccctgatcgcttcacaggcagtggatctgggacagatttcactctcaccatcagcaatgtgcagtctgaagacttggcagagtatttctgtcagcaatataacagctatcctctgacgttcggtggcggcaccaagctggaaatcaaacgggctgccgcagaaggtggaggcggttcaggtggcggaggttccggcggaggtggctctggcggtggcggatcggccatggcccaggtgaagctgcagcagtcaggagggggcttggtgcaacctggaggatccatgaaactctcctgtgttgtctctggattcactttcagtaattactggatgaactgggtccgccagtctccagagaaggggcttgagtggattgcagaaattagattgaaatccaataattttggaagatattatgcggagtctgtgaaagggaggttcaccatctcaagagatgattccaaaagtagtgcctacctgcaaatgatcaacctaagagctgaagatactggcatttattactgtaccagttatggtaactacgttgggcactattttgaccactggggccaagggaccacggtcaccgtatcgagtgccgcggttctagagctcttgagcaactccatcatgtacttcagccacttcgtgccggtcttcctgccagcgaagcccaccacgacgccagcgccgcgaccaccaacaccggcgcccaccatcgcgtcgcagcccctgtccctgcgcccagaggcgtgccggccagcggcggggggcgcagtgcacacgagggggctggacctgctggatcccaaactctgctacctgctggatggaatcctcttcatctatggtgtcattctcactgccttgttcctgagagtgaagttcagcaggagcgcagacgcccccgcgtaccagcagggccagaaccagctctataacgagctcaatctaggacgaagagaggagtacgatgttttggacaagagacgtggccgggaccctgagatggggggaaagccgcagagaaggaagaaccctcaggaaggcctgtacaatgaactgcagaaagataagatggcggaggcctacagtgagattgggatgaaaggcgagcgccggaggggcaaggggcacgatggcctttaccagggtctcagtacagccaccaaggacacctacgacgcccttcacatgcaggccctgccccctcgctaacagccagggcatttctccctcgagcggccgc

SEQ ID NO: 13 - protein, 486 aa, synthetic construct
  REGION 1..486: note = synthetic CSPG4-CAR amino acid sequence
MDWIWRILFLVGAATGAHSAQPADIELTQSPKFMSTSVGDRVSVTCKASQNVDTNVAWYQQKPGQSPEPLLFSASYRYTGVPDRFTGSGSGTDFTLTISNVQSEDLAEYFCQQYNSYPLTFGGGTKLEIKRAAAEGGGGSGGGGSGGGGSGGGGSAMAQVKLQQSGGGLVQPGGSMKLSCVVSGFTFSNYWMNWVRQSPEKGLEWIAEIRLKSNNFGRYYAESVKGRFTISRDDSKSSAYLQMINLRAEDTGIYYCTSYGNYVGHYFDHWGQGTTVTVSSAAVLELLSNSIMYFSHFVPVFLPAKPTTTPAPRPPTPAPTIASQPLSLRPEACRPAAGGAVHTRGLDLLDPKLCYLLDGILFIYGVILTALFLRVKFSRSADAPAYQQGQNQLYNELNLGRREEYDVLDKRRGRDPEMGGKPQRRKNPQEGLYNELQKDKMAEAYSEIGMKGERRRGKGHDGLYQGLSTATKDTYDALHMQALPPR